European Patent Specification EP 3 470 517 B1, published January 10, 2024. Title: Variant Alkaline Protease. Applicant: Kao Corporation. The sequence listing filed with the application follows.

SEQUENCE LISTING (13 sequences)

SEQ ID NO: 1 - DNA, 1302 bp, Bacillus sp. KSM-KP43
  Wild-type
aatgatgttgcgcgtggaattgtcaaagcggatgtggctcagagcagctacgggttgtatggacaaggacagatcgtagcggttgccgatacagggcttgatacaggtcgcaatgacagttcgatgcatgaagccttccgcgggaaaattactgcattatatgcattgggacggacgaataatgccaatgatacgaatggtcatggtacgcatgtggctggctccgtattaggaaacggctccactaataaaggaatggcgcctcaggcgaatctagtcttccaatctatcatggatagcggtgggggacttggaggactaccttcgaatctgcaaaccttattcagccaagcatacagtgctggtgccagaattcatacaaactcctggggagcagcagtgaatggggcttacacaacagattccagaaatgtggatgactatgtgcgcaaaaatgatatgacgatccttttcgctgccgggaatgaaggaccgaacggcggaaccatcagtgcaccaggcacagctaaaaatgcaataacagtcggagctacggaaaacctccgcccaagctttgggtcttatgcggacaatatcaaccatgtggcacagttctcttcacgtggaccgacaaaggatggacggatcaaaccggatgtcatggcaccgggaacgttcatactatcagcaagatcttctcttgcaccggattcctccttctgggcgaaccatgacagtaaatatgcatacatgggtggaacgtccatggctacaccgatcgttgctggaaacgtggcacagcttcgtgagcattttgtgaaaaacagaggcatcacaccaaagccttctctattaaaagcggcactgattgccggtgcagctgacatcggccttggctacccgaacggtaaccaaggatggggacgagtgacattggataaatccctgaacgttgcctatgtgaacgagtccagttctctatccaccagccaaaaagcgacgtactcgtttactgctactgccggcaagcctttgaaaatctccctggtatggtctgatgcccctgcgagcacaactgcttccgtaacgcttgtcaatgatctggaccttgtcattaccgctccaaatggcacacagtatgtaggaaatgactttacttcgccatacaatgataactgggatggccgcaataacgtagaaaatgtatttattaatgcaccacaaagcgggacgtatacaattgaggtacaggcttataacgtaccggttggaccacagaccttctcgttggcaattgtgaat

SEQ ID NO: 2 - protein, 434 aa, Bacillus sp. KSM-KP43
  Wild-type
NDVARGIVKADVAQSSYGLYGQGQIVAVADTGLDTGRNDSSMHEAFRGKITALYALGRTNNANDTNGHGTHVAGSVLGNGSTNKGMAPQANLVFQSIMDSGGGLGGLPSNLQTLFSQAYSAGARIHTNSWGAAVNGAYTTDSRNVDDYVRKNDMTILFAAGNEGPNGGTISAPGTAKNAITVGATENLRPSFGSYADNINHVAQFSSRGPTKDGRIKPDVMAPGTFILSARSSLAPDSSFWANHDSKYAYMGGTSMATPIVAGNVAQLREHFVKNRGITPKPSLLKAALIAGAADIGLGYPNGNQGWGRVTLDKSLNVAYVNESSSLSTSQKATYSFTATAGKPLKISLVWSDAPASTTASVTLVNDLDLVITAPNGTQYVGNDFTSPYNDNWDGRNNVENVFINAPQSGTYTIEVQAYNVPVGPQTFSLAIVN

SEQ ID NO: 3 - protein, 434 aa, Bacillus sp. KSM-KP43
  Valiant
NDVARGIVKADVAQSSYGLYGQGQIVAVADTGLDTGRNDSSMHEAFRGKITALYALGRTNNANDTNGHGTHVAGSVLGNGSTNKGMAPQANLVFQSIMDSGGGLGGLPSNLQTLFSQAYSAGARIHTNSWGTAVNGAYTTDSRNVDDYVRKNDMTILFAAGNEGPNGGTISAPGTAKNAITVGATENLRPSFGSYADNINHVAQFSSRGPTKDGRIKPDVMAPGTFILSARSSLAPDSSFWANHDSKYAYMGGTSMATPIVAGNVAQLREHFVKNRGITPKPSLLKAALIAGAADIGLGYPNGNQGWGRVTLDKSLNVAYVNESSSLSTSQKATYSFTATAGKPLKISLVWSDAPASTTASVTLVNDLDLVITAPNGTQYVGNDFTSPYNDNWDGRNNVENVFINAPQSGTYTIEVQAYNVPVGPQTFSLAIVN

SEQ ID NO: 4 - protein, 434 aa, Bacillus sp. KSM-KP43
  Valiant
NDVARGIVKADVAQSVYGLYGQGQIVAVADTGLDTGRNDSSMHEAFRGKITALYALGRTNNANDPNGHGTHVAGSVLGNGSTAKGMAPQANLVFQSIMDSGGGLGGLPSNLQTLFSQAYSAGARIHTNSWGAAVNGAYTTDSRNVDDYVRKNDMTILFAAGNEGPGVGTISAPGTAKNAITVGATENLRPSFGSQADNINHVAQFSSRGPTKDGRIKPDVMAPGTFILSARSSLAPDSSFWANHDSKYAYMGGTSMATPIVAGNVAQLREHFIKNRGITPKPSLLKAALIAGAADIGLGYPNGNQGWGRVTLDKSLNVAYVNESSSLSTSQKATYSFTATAGKPLKISLVWSDAPASTSASVTLVNDLNLVITAPNGTQYVGNDFTAPYNDNWDGRNNVENVFINAPQSGTYTIEVQAYNVPVGPQTFSLAIVN

SEQ ID NO: 5 - protein, 434 aa, Bacillus sp. KSM-KP43
  Valiant
NDVARGIVKADVAQSVYGLYGQGQIVAVADTGLDTGRNDSSMHEAFRGKITALYALGRTNNANDPNGHGTHVAGSVLGNGSTAKGMAPQANLVFQSIMDSGGGLGGLPSNLQTLFSQAYSAGARIHTNSWGTAVNGAYTTDSRNVDDYVRKNDMTILFAAGNEGPGVGTISAPGTAKNAITVGATENLRPSFGSQADNINHVAQFSSRGPTKDGRIKPDVMAPGTFILSARSSLAPDSSFWANHDSKYAYMGGTSMATPIVAGNVAQLREHFIKNRGITPKPSLLKAALIAGAADIGLGYPNGNQGWGRVTLDKSLNVAYVNESSSLSTSQKATYSFTATAGKPLKISLVWSDAPASTSASVTLVNDLNLVITAPNGTQYVGNDFTAPYNDNWDGRNNVENVFINAPQSGTYTIEVQAYNVPVGPQTFSLAIVN

SEQ ID NO: 6 - protein, 435 aa, Bacillus sp. KSM-KP43
  Valiant
NDVARGIVKADVAQSSYGLYGQGQIVAVADTGLDTGRNDSSMHEAFRGKITALYALGRTNNANDPNGHGTHVAGSVLGNGSTNKGMAPQANLVFQSIMDSGGGLGGLPSNLQTLFSQAYSAGARIHTNSWGASSTNGAYTTDSRNVDDYVRKNDMTILFAAGNEGPGVGTISAPGTAKNAITVGATENLRPSFGSQADNINHVAQFSSRGPTKDGRIKPDVMAPGTFILSARSSLAPDSSFWANHDSKYAYMGGTSMATPIVAGNVAQLREHFIKNRGITPKPSLLKAALIAGAADIGLGYPNGNQGWGRVTLDKSLNVAYVNESSSLSTSQKATYSFTATAGKPLKISLVWSDAPASTSASVTLVNDLNLVITAPNGTQYVGNDFTAPYNDNWDGRNNVENVFINAPQSGTYTIEVQAYNVPVGPQTFSLAIVN

SEQ ID NO: 7 - protein, 435 aa, Bacillus sp. KSM-KP43
  Valiant
NDVARGIVKADVAQSSYGLYGQGQIVAVADTGLDTGRNDISMHEAFRGKITALYALGRVNNANDPNGHGTHVAGSVLGNGLTNKGMAPQANLVFQSIMDSGGGLGGLPSNLQTLFSQAYSAGARIHTNSWGASSTNGAYTTDSRNVDDYVRKNDMTILFAAGNEGPGVGTISAPGTAKNAITVGATENLRPLFGSQADNINHVAQFSSRGPTKDGRIKPDVMAPGTFILSARSSLAPDSSFWANHDSKYAYMGGTSMATPIVAGNVAQLREHFIKNRGITPKPSLLKAALIAGAADIGLGYPNGNQGWGRVTLDKSLNVAYVNESSSLSTSQKATYSFTATAGKPLKISLVWSDAPASTSASVTLVNDLNLVITAPNGTQYVGNDFTAPYNDNWDGRNNVENVFILAPQSGTYTIEVQAYNVPVGPQTFSLAIVN

SEQ ID NO: 8 - protein, 434 aa, Bacillus sp. KSM-KP43
  Valiant
NDVARGIVKADVAQSSYGLYGQGQIVAVADTGLDTGRNDSSMHEAFRGKITALYALGRTNNANDPNGHGTHVAGSVLGNGSTAKGMAPQANLVFQSIMDSGGGLGGLPSNLQTLFSQAYSAGARIHTNSWGTAVNGAYTTDSRNVDDYVRKNDMTILFAAGNEGPGVGTISAPGTAKNAITVGATENLRPSFGSRADNINHVAQFSSRGPTKDGRIKPDVMAPGTFILSARSSLAPDSSFWANHDSKYAYMGGTSMATPIVAGNVAQLREHFIKNRGITPKPSLLKAALIAGAADIGLGYPNGNQGWGRVTLDKSLNVAYVNESSSLSTSQKATYSFTATAGKPLKISLVWSDAPASTSASVTLVNDLNLVITAPNGTQYVGNDFTAPYNDNWDGRNNVENVFINAPQSGTYTIEVQAYNVPVGPQTFSLAIVN

SEQ ID NO: 9 - protein, 435 aa, Bacillus sp. KSM-KP43
  Valiant
NDVARGIVKADVAQSSYGLYGQGQIVAVADTGLDTGRNDSSMHEAFRGKITALYALGRTNNANDPNGHGTHVAGSVLGNGSTNKGMAPQANLVFQSIMDSGGGLGGLPSNLQTLFSQAYSAGARIHTNSWGASSTNGAYTTDSRNVDDYVRKNDMTILFAAGNEGPGVGTISAPGTAKNAITVGATENLRPSFGSRADNINHVAQFSSRGPTKDGRIKPDVMAPGTFILSARSSLAPDSSFWANHDSKYAYMGGTSMATPIVAGNVAQLREHFIKNRGITPKPSLLKAALIAGAADIGLGYPNGNQGWGRVTLDKSLNVAYVNESSSLSTSQKATYSFTATAGKPLKISLVWSDAPASTSASVTLVNDLNLVITAPNGTQYVGNDFTAPYNDNWDGRNNVENVFINAPQSGTYTIEVQAYNVPVGPQTFSLAIVN

SEQ ID NO: 10 - protein, 434 aa, Bacillus sp. KSM-KP43
  Valiant
NDVARGIVKADVAQSVYGLYGQGQIVAVADTGLDTGRNDSSMHEAFRGKITALYALGRTNNANDPNGHGTHVAGSVLGNGSTAKGMAPQANLVFQSIMDSGGGLGGLPSNLQTLFSQAYSAGARIHTNSWGAAVNGAYTTDSRNVDDYVRKNDMTILFAAGNEGPGVGTISAPGTAKNAITVGATENLRPSFGSQADNINHVADFSSRGPTKDGRIKPDVMAPGTFILSARSSLAPDSSFWANHDSKYAYMGGTSMATPIVAGNVAQLREHFIKNRGITPKPSLLKAALIAGAADIGLGYPNGNQGWGRVTLDKSLNVVYVNESSSLSTSQKATYSFTATAGKPLKISLVWSDAPASTSASVTLVNDLNLVITAPNGTQYVGNDFTAPYNDNWDGRNNVENVFINAPQSGTYTIEVQAYNVPVGPQTFSLAIVN

SEQ ID NO: 11 - protein, 435 aa, Bacillus sp. KSM-KP43
  Valiant
NDVARGIVKADVAQSSYGLYGQGQIVAVADTGLDTGRNDSSMHEAFRGKITALYALGRTNNANDPNGHGTHVAGSVLGNGSTNKGMAPQANLVFQSIMDSGGGLGGLPSNLQTLFSQAYSAGARIHTNSWGASSTNGAYTTDSRNVDDYVRKNDMTILFAAGNEGPGVGTISAPGTAKNAITVGATENLRPSFGRRADNINHVAQFSSRGPTRDGRIKPDVMAPGTFILSARSSLAPDSSFWANHDSKYAYMGGTSMATPIVAGNVAQLREHFIKNRGITPKPSLLKAALIAGAADIGLGYPNGNQGWGRVTLDKSLNVAYVNESSSLSTSQKATYSFTATAGKPLKISLVWSDAPASTSASVTLVNDLNLVITAPNGTRYVGNDFTAPYNDNWDGRNNVENVFINAPQSGTYTIEVQAYNVPVGPQTFSLAIVN

SEQ ID NO: 12 - DNA, 27 bp, Artificial
  Oligonucleotide primer A294-F
ggtgcaactgacatcggccttggctac

SEQ ID NO: 13 - DNA, 27 bp, Artificial
  Oligonucleotide primer A294-R
gatgtcagttgcaccggcaatcagtgc